European Patent Application EP 4 585 685 A1, published July 16, 2025. Title: CONSTRUCT COMPRISING UTR SEQUENCE THAT IMPROVES INTRACELLULAR STABILITY AND BIOSYNTHESIS OF MRNA AND USE THEREOF. Applicant: 주식회사 테라젠바이오. Application US. The sequence listing filed with the application follows.

SEQUENCE LISTING (37 sequences)

SEQ ID NO: 1 - DNA, 37 bp, Homo sapiens
  source 1..37: mol_type = genomic DNA
aaaccataccatatcccaccagagagtcgcagccacc

SEQ ID NO: 2 - RNA, 37 nt, Homo sapiens
  source 1..37: mol_type = mRNA
aaaccataccatatcccaccagagagtcgcagccacc

SEQ ID NO: 3 - DNA, 24 bp, Homo sapiens
  source 1..24: mol_type = genomic DNA
gtcctgtggcctctgcaggccacc

SEQ ID NO: 4 - RNA, 24 nt, Homo sapiens
  source 1..24: mol_type = mRNA
gtcctgtggcctctgcaggccacc

SEQ ID NO: 5 - DNA, 42 bp, Homo sapiens
  source 1..42: mol_type = genomic DNA
agaagtgtctgacaaaacaaagaaacaaaacctcaggccacc

SEQ ID NO: 6 - RNA, 42 nt, Homo sapiens
  source 1..42: mol_type = mRNA
agaagtgtctgacaaaacaaagaaacaaaacctcaggccacc

SEQ ID NO: 7 - DNA, 35 bp, Homo sapiens
  source 1..35: mol_type = genomic DNA
gtctcccgccacccacaccagctgtcccagccacc

SEQ ID NO: 8 - RNA, 35 nt, Homo sapiens
  source 1..35: mol_type = mRNA
gtctcccgccacccacaccagctgtcccagccacc

SEQ ID NO: 9 - DNA, 47 bp, Homo sapiens
  source 1..47: mol_type = genomic DNA
ctgctcagttcatccctagaggcagctgctccaggaacagagccacc

SEQ ID NO: 10 - RNA, 47 nt, Homo sapiens
  source 1..47: mol_type = mRNA
ctgctcagttcatccctagaggcagctgctccaggaacagagccacc

SEQ ID NO: 11 - DNA, 26 bp, Homo sapiens
  source 1..26: mol_type = genomic DNA
agcaagctgtcctgtgagccgccacc

SEQ ID NO: 12 - RNA, 26 nt, Homo sapiens
  source 1..26: mol_type = mRNA
agcaagctgtcctgtgagccgccacc

SEQ ID NO: 13 - DNA, 29 bp, Homo sapiens
  source 1..29: mol_type = genomic DNA
gcagtcgccacacctttgcccctgccacc

SEQ ID NO: 14 - RNA, 29 nt, Homo sapiens
  source 1..29: mol_type = mRNA
gcagtcgccacacctttgcccctgccacc

SEQ ID NO: 15 - DNA, 42 bp, Homo sapiens
  source 1..42: mol_type = genomic DNA
ccgctgaagtggagcaggtacagtcacagctgtggggccacc

SEQ ID NO: 16 - RNA, 42 nt, Homo sapiens
  source 1..42: mol_type = mRNA
ccgctgaagtggagcaggtacagtcacagctgtggggccacc

SEQ ID NO: 17 - DNA, 24 bp, Homo sapiens
  source 1..24: mol_type = genomic DNA
ggcggccgcgcggaggaggccacc

SEQ ID NO: 18 - RNA, 24 nt, Homo sapiens
  source 1..24: mol_type = mRNA
ggcggccgcgcggaggaggccacc

SEQ ID NO: 19 - DNA, 52 bp, Homo sapiens
  source 1..52: mol_type = genomic DNA
gaataaactagtattcttctggtccccacagactcagagagaacccgccacc

SEQ ID NO: 20 - DNA, 219 bp, Homo sapiens
  source 1..219: mol_type = genomic DNA
tgcaggagggaagtcagcagcctgtgtttggtgtgcaactcatcatgggcatgagaccagtgtgaggactcaccctggaagagaatattcgcttaattcccccaacctgaccacctcattcttatctttcttctgtttcttcctccccgctgtcatttcagtctcttcattttgtcatacggcctaaggctttaaagagcaataaaatttttagtctgc

SEQ ID NO: 21 - RNA, 219 nt, Homo sapiens
  source 1..219: mol_type = mRNA
tgcaggagggaagtcagcagcctgtgtttggtgtgcaactcatcatgggcatgagaccagtgtgaggactcaccctggaagagaatattcgcttaattcccccaacctgaccacctcattcttatctttcttctgtttcttcctccccgctgtcatttcagtctcttcattttgtcatacggcctaaggctttaaagagcaataaaatttttagtctgc

SEQ ID NO: 22 - DNA, 162 bp, Homo sapiens
  source 1..162: mol_type = genomic DNA
ggggccttctgacatgagtctggcctggccccacctcctagttcctcataataaagacagattgcttcttcgcttctcactgaggggccttctgacatgagtctggcctggccccacctccccagtttctcataataaagacagattgcttcttcacttgaa

SEQ ID NO: 23 - RNA, 162 nt, Homo sapiens
  source 1..162: mol_type = mRNA
ggggccttctgacatgagtctggcctggccccacctcctagttcctcataataaagacagattgcttcttcgcttctcactgaggggccttctgacatgagtctggcctggccccacctccccagtttctcataataaagacagattgcttcttcacttgaa

SEQ ID NO: 24 - DNA, 225 bp, Homo sapiens
  source 1..225: mol_type = genomic DNA
taatttagccaggctatgaaatcatcctgtgagttatttcctccataataaccctgcatttcccattaatctacatatcttcccacagcagctttgctcagtgatacccacatgggaaaaatcccaggggatgttgcttactctttttgcccacactgctttggatacttatctactgtccgaaggccttctttccccactcaattcttcctgccctgttattaa

SEQ ID NO: 25 - RNA, 225 nt, Homo sapiens
  source 1..225: mol_type = mRNA
taatttagccaggctatgaaatcatcctgtgagttatttcctccataataaccctgcatttcccattaatctacatatcttcccacagcagctttgctcagtgatacccacatgggaaaaatcccaggggatgttgcttactctttttgcccacactgctttggatacttatctactgtccgaaggccttctttccccactcaattcttcctgccctgttattaa

SEQ ID NO: 26 - DNA, 164 bp, Homo sapiens
  source 1..164: mol_type = genomic DNA
gactgcccacccactcccacacctagcccagaatgctgtaggccactaggcgcaggggcatctctcccctgctccagcgcatctcccgggctggccacctccttgaccagcatatctgttttctgattgcgctcttcacaattaaaggcctcctgcaaaccttt

SEQ ID NO: 27 - RNA, 164 nt, Homo sapiens
  source 1..164: mol_type = mRNA
gactgcccacccactcccacacctagcccagaatgctgtaggccactaggcgcaggggcatctctcccctgctccagcgcatctcccgggctggccacctccttgaccagcatatctgttttctgattgcgctcttcacaattaaaggcctcctgcaaaccttt

SEQ ID NO: 28 - DNA, 188 bp, Homo sapiens
  source 1..188: mol_type = genomic DNA
gacctcaataccccaagtccacctgcctatccatcctgcgagctccttgggtcctgcaatctccagggctgcccctgtaggttgcttaaaagggacagtattctcagtgctctcctaccccacctcatgcctggcccccctccaggcatgctggcctcccaataaagctggacaagaagctgctatga

SEQ ID NO: 29 - RNA, 188 nt, Homo sapiens
  source 1..188: mol_type = mRNA
gacctcaataccccaagtccacctgcctatccatcctgcgagctccttgggtcctgcaatctccagggctgcccctgtaggttgcttaaaagggacagtattctcagtgctctcctaccccacctcatgcctggcccccctccaggcatgctggcctcccaataaagctggacaagaagctgctatga

SEQ ID NO: 30 - RNA, 175 nt, Homo sapiens
  source 1..175: mol_type = mRNA
atgctgaccttcacccagagctgcctatgcccagcctccaactccagctgagtcctggggttggggagggggtcggggtcccaggacctgagcctggccatgtcctcaaccccaaatcccccgactccctccccagatctgtcctgggggatgcaaataaagcctgctctcccaa

SEQ ID NO: 31 - DNA, 206 bp, Homo sapiens
  source 1..206: mol_type = genomic DNA
tggccggtgagctgcggagagctcatggaaggcgagtgggaacccggctgcctgcctttttttctgatccagaccctcggcacctgctacttaccaactggaaaattttatgcatcccatgaagcccagatacacaaaattccaccccatgatcaagaatcctgctccactaagaatggtgctaaagtaaaactagtttaataagc

SEQ ID NO: 32 - RNA, 206 nt, Homo sapiens
  source 1..206: mol_type = mRNA
tggccggtgagctgcggagagctcatggaaggcgagtgggaacccggctgcctgcctttttttctgatccagaccctcggcacctgctacttaccaactggaaaattttatgcatcccatgaagcccagatacacaaaattccaccccatgatcaagaatcctgctccactaagaatggtgctaaagtaaaactagtttaataagc

SEQ ID NO: 33 - DNA, 210 bp, Homo sapiens
  source 1..210: mol_type = genomic DNA
tcagagaggatggcctgcagccacatgggaggaaggcccaggggtggggcccatggggtctctgcatcttcagtcgtctgtcccaagtcctgctcctttctgcccagcctgctcagcaggttgaatgggttctcagtggtcaccttcctcagctcagctgggccactcctcttcacccaccccatggagacaataaacagctgaaccatg

SEQ ID NO: 34 - RNA, 210 nt, Homo sapiens
  source 1..210: mol_type = mRNA
tcagagaggatggcctgcagccacatgggaggaaggcccaggggtggggcccatggggtctctgcatcttcagtcgtctgtcccaagtcctgctcctttctgcccagcctgctcagcaggttgaatgggttctcagtggtcaccttcctcagctcagctgggccactcctcttcacccaccccatggagacaataaacagctgaaccatg

SEQ ID NO: 35 - DNA, 189 bp, Homo sapiens
  source 1..189: mol_type = genomic DNA
ccctgtccagtgtctgcttgccatcctgccagaacaggccctcaagcccaagagccatcccaggcctgttcaggcctcagctaagcctctcttcatctggaagaagaggcaagggggcaggagaccaggctctagctctgggccctccttcagcccccatcatgggaataaattaattttctcaatgta

SEQ ID NO: 36 - RNA, 189 nt, Homo sapiens
  source 1..189: mol_type = mRNA
ccctgtccagtgtctgcttgccatcctgccagaacaggccctcaagcccaagagccatcccaggcctgttcaggcctcagctaagcctctcttcatctggaagaagaggcaagggggcaggagaccaggctctagctctgggccctccttcagcccccatcatgggaataaattaattttctcaatgta

SEQ ID NO: 37 - DNA, 297 bp, Homo sapiens
  source 1..297: mol_type = genomic DNA
ctcgagctggtactgcatgcacgcaatgctagctgcccctttcccgtcctgggtaccccgagtctcccccgacctcgggtcccaggtatgctcccacctccacctgccccactcaccacctctgctcgttccagacacctcccaagcacgcagcaatgcagctcaaaacgcttagcctagccacacccccacgggaaacagcagtgattaacctttagcaataaacgaaagtttaactaagctatactaaccccagggttggtcaatttcgtgccagccacaccctggagctagcaa